European Patent Application EP 4 198 045 A1, published June 21, 2023. Title: ANTIMICROBIAL PEPTIDES, VARIANTS AND CHEMICAL ANALOGUES THEREOF AND THEIR USES. Applicant: UNIVERSITE DE LILLE/CENTRE NATIONAL DE LA RECHERCHE SCIENTIFIQUE (CNRS)/UNIVERSITE D'AIX MARSEILLE/SORBONNE UNIVERSITE/ECOLE CENTRALE DE MARSEILLE. The sequence listing filed with the application follows.

SEQUENCE LISTING (20 sequences)

SEQ ID NO: 1 - protein, 215 aa, Capitella sp.
  MISC_FEATURE: propeptide
MEKVLIQDQPPKYGAGRTDTKKTCLLMYAVAMTILVFAIMVTGVVMFVLHVDNKVDIDTLPSTVEHYQVNGEDIEQHVLIDDARETEIIRYEDSGAILVLDYRKGLTALYVPSAKECFLTGGIDRNLPSPFHGEVEKNDAIDDGAEVTYRKCNSFPVMDHSVLPPHLTSFCEHKPVFWVVPSNGDQGEQRTKRSPGRVCVRICRNGRCYRRCWNT

SEQ ID NO: 2 - protein, 19 aa, Capitella sp.
  peptide Michelicin
RVCVRICRNGRCYRRCWNT

SEQ ID NO: 3 - protein, 19 aa, Capitella sp.
  variant V1
RVCVRVCRNGRCYRRCWNT

SEQ ID NO: 4 - protein, 19 aa, Capitella sp.
  variant V2
RFCVRVCRNGRCIMKCWNT

SEQ ID NO: 5 - protein, 19 aa, Capitella sp.
  variant V3
RICVRVCRNGRCIMKCWNT

SEQ ID NO: 6 - protein, 19 aa, Capitella sp.
  variant V4
RICVRVCRNGFCFMKCWNT

SEQ ID NO: 7 - protein, 19 aa, Capitella sp.
  variant V5
RFCVRVCLFIRCFMKCWNT

SEQ ID NO: 8 - protein, 19 aa, Capitella sp.
  variant  V6
RICVRVCRNGRCFMKCWNT

SEQ ID NO: 9 - protein, 23 aa, Capitella sp.
  variant V7
RKAVSTCVRVCRNGFCFMKCWNT

SEQ ID NO: 10 - protein, 19 aa, Capitella sp.
  variant V8
RVCVRICRNGFCFMKCWNT

SEQ ID NO: 11 - protein, 19 aa, Capitella sp.
  variant V9
RVCVRVCRNGFCFMKCWNT

SEQ ID NO: 12 - protein, 18 aa, Capitella sp.
  variant V10
RVCIRVCRNGVCYRRCWG

SEQ ID NO: 13 - protein, 19 aa, Artificial
  chemical analogue CA1
KVCVKICKNGKCYKKCWNT

SEQ ID NO: 14 - protein, 6 aa, Artificial
  chemical analogue CA2
CRNGRC

SEQ ID NO: 15 - protein, 9 aa, Artificial
  chemical analogue CA3
CRNGRCYRR

SEQ ID NO: 16 - protein, 11 aa, Artificial
  chemical analogue CA4
RICRNGRCYRR

SEQ ID NO: 17 - protein, 14 aa, Artificial
  chemical analogue CA5
CVRICRNGRCYRRC

SEQ ID NO: 18 - protein, 19 aa, Artificial
  chemical analogue CA6, wherein Xaa=Abu (2-Aminobutanoic group)
  misc_feature (3)..(3): Xaa = Abu
  misc_feature (7)..(7): Xaa = Abu
  misc_feature (12)..(12): Xaa = Abu
  misc_feature (16)..(16): Xaa = Abu
RVXVRIXRNGRXYRRXWNT

SEQ ID NO: 19 - protein, 19 aa, Artificial
  chemical analogue CA7, wherein Xaa=Abu (2-Aminobutanoic group) and having a N terminus linked with a cycle
  misc_feature (3)..(3): Xaa = Abu
  misc_feature (7)..(7): Xaa = Abu
  misc_feature (12)..(12): Xaa = Abu
  misc_feature (16)..(16): Xaa = Abu
RVXVRIXRNGRXYRRXWNT

SEQ ID NO: 20 - DNA, 57 bp, Capitella sp.
  nucleic acid encoding peptide Michelicin
cgcgtctgtgttaggatttgtcgcaatggacggtgctacagaagatgttggaacact